European Patent Application EP 4 269 574 A1, published November 1, 2023. Title: ATP-PRT variant with reduced feedback inhibition by histidine and histidine-producing strain expressing the same. Applicant: Daesang Corporation. The sequence listing filed with the application follows.

SEQUENCE LISTING (53 sequences)

SEQ ID NO: 1 - protein, 299 aa, Artificial Sequence
  hisG_WT
MTDNTRLRIAMQKSGRLSDDSRELLARCGIKINLHTQRLIAMAENMPIDILRVRDDDIPGLVMDGVVDLGIIGENVLEEELLNRRAQGEDPRYFTLRRLDFGGCRLSLATPVDEAWDGPLSLNGKRIATSYPHLLKRYLDQKGISFKSCLLNGSVEVAPRAGLADAICDLVSTGATLEANGLREVEVIYRSKACLIQRDGEMEESKQQLIDKLLTRIQGVIQARESKYIMMHAPTERLDEVIALLPGAERPTILPLAGDQQRVAMHMVSSETLFWETMEKLKALGASSILVLPIEKMME

SEQ ID NO: 2 - protein, 299 aa, Artificial Sequence
  hisG_H232K/T
  VARIANT (232): Xaa (232) = K or T
MTDNTRLRIAMQKSGRLSDDSRELLARCGIKINLHTQRLIAMAENMPIDILRVRDDDIPGLVMDGVVDLGIIGENVLEEELLNRRAQGEDPRYFTLRRLDFGGCRLSLATPVDEAWDGPLSLNGKRIATSYPHLLKRYLDQKGISFKSCLLNGSVEVAPRAGLADAICDLVSTGATLEANGLREVEVIYRSKACLIQRDGEMEESKQQLIDKLLTRIQGVIQARESKYIMMXAPTERLDEVIALLPGAERPTILPLAGDQQRVAMHMVSSETLFWETMEKLKALGASSILVLPIEKMME

SEQ ID NO: 3 - protein, 299 aa, Artificial Sequence
  hisG_R250H
MTDNTRLRIAMQKSGRLSDDSRELLARCGIKINLHTQRLIAMAENMPIDILRVRDDDIPGLVMDGVVDLGIIGENVLEEELLNRRAQGEDPRYFTLRRLDFGGCRLSLATPVDEAWDGPLSLNGKRIATSYPHLLKRYLDQKGISFKSCLLNGSVEVAPRAGLADAICDLVSTGATLEANGLREVEVIYRSKACLIQRDGEMEESKQQLIDKLLTRIQGVIQARESKYIMMHAPTERLDEVIALLPGAEHPTILPLAGDQQRVAMHMVSSETLFWETMEKLKALGASSILVLPIEKMME

SEQ ID NO: 4 - protein, 299 aa, Artificial Sequence
  hisG_T252A/L
  VARIANT (252): Xaa (252) = A or L
MTDNTRLRIAMQKSGRLSDDSRELLARCGIKINLHTQRLIAMAENMPIDILRVRDDDIPGLVMDGVVDLGIIGENVLEEELLNRRAQGEDPRYFTLRRLDFGGCRLSLATPVDEAWDGPLSLNGKRIATSYPHLLKRYLDQKGISFKSCLLNGSVEVAPRAGLADAICDLVSTGATLEANGLREVEVIYRSKACLIQRDGEMEESKQQLIDKLLTRIQGVIQARESKYIMMHAPTERLDEVIALLPGAERPXILPLAGDQQRVAMHMVSSETLFWETMEKLKALGASSILVLPIEKMME

SEQ ID NO: 5 - protein, 299 aa, Artificial Sequence
  hisG_E271K
MTDNTRLRIAMQKSGRLSDDSRELLARCGIKINLHTQRLIAMAENMPIDILRVRDDDIPGLVMDGVVDLGIIGENVLEEELLNRRAQGEDPRYFTLRRLDFGGCRLSLATPVDEAWDGPLSLNGKRIATSYPHLLKRYLDQKGISFKSCLLNGSVEVAPRAGLADAICDLVSTGATLEANGLREVEVIYRSKACLIQRDGEMEESKQQLIDKLLTRIQGVIQARESKYIMMHAPTERLDEVIALLPGAERPTILPLAGDQQRVAMHMVSSKTLFWETMEKLKALGASSILVLPIEKMME

SEQ ID NO: 6 - protein, 299 aa, Artificial Sequence
  hisG_S288P
MTDNTRLRIAMQKSGRLSDDSRELLARCGIKINLHTQRLIAMAENMPIDILRVRDDDIPGLVMDGVVDLGIIGENVLEEELLNRRAQGEDPRYFTLRRLDFGGCRLSLATPVDEAWDGPLSLNGKRIATSYPHLLKRYLDQKGISFKSCLLNGSVEVAPRAGLADAICDLVSTGATLEANGLREVEVIYRSKACLIQRDGEMEESKQQLIDKLLTRIQGVIQARESKYIMMHAPTERLDEVIALLPGAERPTILPLAGDQQRVAMHMVSSETLFWETMEKLKALGASPILVLPIEKMME

SEQ ID NO: 7 - protein, 299 aa, Artificial Sequence
  hisG_SDM4
MTDNTRLRIAMQKSGRLSDDSRELLARCGIKINLHTQRLIAMAENMPIDILRVRDDDIPGLVMDGVVDLGIIGENVLEEELLNRRAQGEDPRYFTLRRLDFGGCRLSLATPVDEAWDGPLSLNGKRIATSYPHLLKRYLDQKGISFKSCLLNGSVEVAPRAGLADAICDLVSTGATLEANGLREVEVIYRSKACLIQRDGEMEESKQQLIDKLLTRIQGVIQARESKYIMMKAPTERLDEVIALLPGAERPAILPLAGDQQRVAMHMVSSKTLFWETMEKLKALGASPILVLPIEKMME

SEQ ID NO: 8 - protein, 299 aa, Artificial Sequence
  hisG_SDM7
MTDNTRLRIAMQKSGRLSDDSRELLARCGIKINLHTQRLIAMAENMPIDILRVRDDDIPGLVMDGVVDLGIIGENVLEEELLNRRAQGEDPRYFTLRRLDFGGCRLSLATPVDEAWDGPLSLNGKRIATSYPHLLKRYLDQKGISFKSCLLNGSVEVAPRAGLADAICDLVSTGATLEANGLREVEVIYRSKACLIQRDGEMEESKQQLIDKLLTRIQGVIQARESKYIMMTAPTERLDEVIALLPGAEHPLILPLAGDQQRVAMHMVSSKTLFWETMEKLKALGASPILVLPIEKMME

SEQ ID NO: 9 - DNA, 23 bp, Artificial Sequence
  hisGW_CF
agttcattgtacaatgatgagcg

SEQ ID NO: 10 - DNA, 20 bp, Artificial Sequence
  hisGW_CR
agccgccaggaatatacaac

SEQ ID NO: 11 - DNA, 28 bp, Artificial Sequence
  232K-R
tttcatcatgatgtattttgattcgcgc

SEQ ID NO: 12 - DNA, 28 bp, Artificial Sequence
  232K-F
gcgcgaatcaaaatacatcatgatgaaa

SEQ ID NO: 13 - DNA, 28 bp, Artificial Sequence
  232E-R
ttccatcatgatgtattttgattcgcgc

SEQ ID NO: 14 - DNA, 28 bp, Artificial Sequence
  232E-F
gcgcgaatcaaaatacatcatgatggaa

SEQ ID NO: 15 - DNA, 22 bp, Artificial Sequence
  240K-R
tttatccagacgttcggtcggt

SEQ ID NO: 16 - DNA, 22 bp, Artificial Sequence
  240K-F
accgaccgaacgtctggataaa

SEQ ID NO: 17 - DNA, 20 bp, Artificial Sequence
  248F-R
gaaacctggcagcagggcga

SEQ ID NO: 18 - DNA, 20 bp, Artificial Sequence
  248F-F
tcgccctgctgccaggtttc

SEQ ID NO: 19 - DNA, 20 bp, Artificial Sequence
  252A-R
cccgccagcggcagaatcgc

SEQ ID NO: 20 - DNA, 20 bp, Artificial Sequence
  252A-F
gcgattctgccgctggcggg

SEQ ID NO: 21 - DNA, 25 bp, Artificial Sequence
  250H-R
ccgccagcggcagaatagttggatg

SEQ ID NO: 22 - DNA, 25 bp, Artificial Sequence
  250H-F
catccaactattctgccgctggcgg

SEQ ID NO: 23 - DNA, 25 bp, Artificial Sequence
  250E-R
ccgccagcggcagaatagttggttc

SEQ ID NO: 24 - DNA, 25 bp, Artificial Sequence
  250E-F
gaaccaactattctgccgctggcgg

SEQ ID NO: 25 - DNA, 25 bp, Artificial Sequence
  252L-R
ccgccagcggcagaatcaatgggcg

SEQ ID NO: 26 - DNA, 25 bp, Artificial Sequence
  252L-F
cgcccattgattctgccgctggcgg

SEQ ID NO: 27 - DNA, 25 bp, Artificial Sequence
  252P-R
ccgccagcggcagaatcggtgggcg

SEQ ID NO: 28 - DNA, 25 bp, Artificial Sequence
  252P-F
cgcccaccgattctgccgctggcgg

SEQ ID NO: 29 - DNA, 25 bp, Artificial Sequence
  252Q-R
ccgccagcggcagaatctgtgggcg

SEQ ID NO: 30 - DNA, 25 bp, Artificial Sequence
  252Q-F
cgcccacagattctgccgctggcgg

SEQ ID NO: 31 - DNA, 20 bp, Artificial Sequence
  271K-R
tttgctgctgaccatgtgca

SEQ ID NO: 32 - DNA, 20 bp, Artificial Sequence
  271K-F
tgcacatggtcagcagcaaa

SEQ ID NO: 33 - DNA, 23 bp, Artificial Sequence
  288P-R
cggactggcacccagcgctttca

SEQ ID NO: 34 - DNA, 23 bp, Artificial Sequence
  288P-F
tgaaagcgctgggtgccagtccg

SEQ ID NO: 35 - DNA, 23 bp, Artificial Sequence
  288K-R
cttactggcacccagcgctttca

SEQ ID NO: 36 - DNA, 23 bp, Artificial Sequence
  288K-F
tgaaagcgctgggtgccagtaag

SEQ ID NO: 37 - DNA, 28 bp, Artificial Sequence
  232T-R
tgtcatcatgatgtattttgattcgcgc

SEQ ID NO: 38 - DNA, 28 bp, Artificial Sequence
  232T-F
gcgcgaatcaaaatacatcatgatgaca

SEQ ID NO: 39 - DNA, 26 bp, Artificial Sequence
  hisG_HF-F
gctcattcattaaacaaatccattgc

SEQ ID NO: 40 - DNA, 25 bp, Artificial Sequence
  hisG_HF-R
tttgttattcctctttaaacctgtc

SEQ ID NO: 41 - DNA, 40 bp, Artificial Sequence
  FR(hisG)-F
gtttaaagaggaataacaaagtgtaggctggagctgcttc

SEQ ID NO: 42 - DNA, 41 bp, Artificial Sequence
  FR(hisG)-R
ccagatcaattcgcgctaactctgtcaaacatgagaattaa

SEQ ID NO: 43 - DNA, 41 bp, Artificial Sequence
  hisG+FR-F
ttaattctcatgtttgacagagttagcgcgaattgatctgg

SEQ ID NO: 44 - DNA, 43 bp, Artificial Sequence
  hisG+HR-R
tgtgttaaagctcatggcgatcactccatcatcttctcaatcg

SEQ ID NO: 45 - DNA, 21 bp, Artificial Sequence
  hisG_HR-F
tcgccatgagctttaacacaa

SEQ ID NO: 46 - DNA, 24 bp, Artificial Sequence
  hisG_HR-R
agtgtggaaggtttcaatattctt

SEQ ID NO: 47 - DNA, 33 bp, Artificial Sequence
  hisG-F
atatgaattcatgacagacaacactcgtttacg

SEQ ID NO: 48 - DNA, 49 bp, Artificial Sequence
  hisG-R
atataagctttcactccatcatcttctcaatcggcaggaccagaatcgg

SEQ ID NO: 49 - DNA, 45 bp, Artificial Sequence
  271K-R2
atatagcgctttcagtttttccatggtttcccagaacagggtttt

SEQ ID NO: 50 - DNA, 25 bp, Artificial Sequence
  hisG-CF
atattctgaaatgagctgttgacaa

SEQ ID NO: 51 - DNA, 20 bp, Artificial Sequence
  hisG-CR
tactgccgccaggcaaattc

SEQ ID NO: 52 - DNA, 25 bp, Artificial Sequence
  250H+252L-R
ccgccagcggcagaatcaatggatg

SEQ ID NO: 53 - DNA, 25 bp, Artificial Sequence
  250H+252L-F
catccattgattctgccgctggcgg